European Patent Specification EP 3 745 862 B1, published June 26, 2024. Title: Methods of Treating Fibrotic Pathologies. Applicant: Mayo Foundation for Medical Education and Research. The sequence listing filed with the application follows.

SEQUENCE LISTING (54 sequences)

SEQ ID NO: 1 - DNA, 22 bp, Artificial Sequence
  synthetically generated oligonucleotide
cccagccctatcagtcatattg

SEQ ID NO: 2 - DNA, 21 bp, Artificial Sequence
  synthetically generated oligonucleotide
aggattcatctgcgagttcag

SEQ ID NO: 3 - DNA, 17 bp, Artificial Sequence
  synthetically generated oligonucleotide
gtccagcacgaggctca

SEQ ID NO: 4 - DNA, 17 bp, Artificial Sequence
  synthetically generated oligonucleotide
tcgccttcgtggtcctc

SEQ ID NO: 5 - DNA, 23 bp, Artificial Sequence
  synthetically generated oligonucleotide
aagggacacagaggtttcagtgg

SEQ ID NO: 6 - DNA, 24 bp, Artificial Sequence
  synthetically generated oligonucleotide
cagcaccagtagcaccatcatttc

SEQ ID NO: 7 - DNA, 21 bp, Artificial Sequence
  synthetically generated oligonucleotide
gtgaagaagaggacagcactg

SEQ ID NO: 8 - DNA, 18 bp, Artificial Sequence
  synthetically generated oligonucleotide
cccattcccaccatcacc

SEQ ID NO: 9 - DNA, 20 bp, Artificial Sequence
  synthetically generated oligonucleotide
tgtcagtcaaagcaagcccg

SEQ ID NO: 10 - DNA, 24 bp, Artificial Sequence
  synthetically generated oligonucleotide
ttaggacgctcataagtgtcaccc

SEQ ID NO: 11 - DNA, 21 bp, Artificial Sequence
  synthetically generated oligonucleotide
tcagctacaatgggatcttgg

SEQ ID NO: 12 - DNA, 21 bp, Artificial Sequence
  synthetically generated oligonucleotide
aaggcagtcacggtatttctc

SEQ ID NO: 13 - DNA, 21 bp, Artificial Sequence
  synthetically generated oligonucleotide
acattcgctacacaggacatc

SEQ ID NO: 14 - DNA, 20 bp, Artificial Sequence
  synthetically generated oligonucleotide
ttcccacttcagaacaccag

SEQ ID NO: 15 - DNA, 20 bp, Artificial Sequence
  synthetically generated oligonucleotide
tgccagtggatcgacataac

SEQ ID NO: 16 - DNA, 21 bp, Artificial Sequence
  synthetically generated oligonucleotide
gaaacgtagcgacctgtgtag

SEQ ID NO: 17 - DNA, 20 bp, Artificial Sequence
  synthetically generated oligonucleotide
gtgcagcgacaaaaggattc

SEQ ID NO: 18 - DNA, 19 bp, Artificial Sequence
  synthetically generated oligonucleotide
gcggtaggttgagaggatg

SEQ ID NO: 19 - DNA, 19 bp, Artificial Sequence
  synthetically generated oligonucleotide
agcgaaaagagggtcaacg

SEQ ID NO: 20 - DNA, 22 bp, Artificial Sequence
  synthetically generated oligonucleotide
tgtcattggcacgatagaactc

SEQ ID NO: 21 - DNA, 21 bp, Artificial Sequence
  synthetically generated oligonucleotide
gtggcagagtcagatttctcc

SEQ ID NO: 22 - DNA, 20 bp, Artificial Sequence
  synthetically generated oligonucleotide
ttgttcctgagacgctgttc

SEQ ID NO: 23 - DNA, 21 bp, Artificial Sequence
  synthetically generated oligonucleotide
gggagatgaagtttgaggtgg

SEQ ID NO: 24 - DNA, 21 bp, Artificial Sequence
  synthetically generated oligonucleotide
agatggtctgtatagtccggg

SEQ ID NO: 25 - DNA, 22 bp, Artificial Sequence
  synthetically generated oligonucleotide
aaacccagatcgagactcaaag

SEQ ID NO: 26 - DNA, 20 bp, Artificial Sequence
  synthetically generated oligonucleotide
acccattcccaaagtagcag

SEQ ID NO: 27 - DNA, 23 bp, Artificial Sequence
  synthetically generated oligonucleotide
ctccttccagttttacagcaaag

SEQ ID NO: 28 - DNA, 19 bp, Artificial Sequence
  synthetically generated oligonucleotide
tttccccagttttctcccc

SEQ ID NO: 29 - DNA, 21 bp, Artificial Sequence
  synthetically generated oligonucleotide
tgcctaccgacaagattgatg

SEQ ID NO: 30 - DNA, 21 bp, Artificial Sequence
  synthetically generated oligonucleotide
atcccttcccagactttgatg

SEQ ID NO: 31 - DNA, 21 bp, Artificial Sequence
  synthetically generated oligonucleotide
cccgtagccattatgatcgtc

SEQ ID NO: 32 - DNA, 20 bp, Artificial Sequence
  synthetically generated oligonucleotide
agagcattcgacagggtttc

SEQ ID NO: 33 - DNA, 21 bp, Artificial Sequence
  synthetically generated oligonucleotide
tccttctaccacctcagcgag

SEQ ID NO: 34 - DNA, 23 bp, Artificial Sequence
  synthetically generated oligonucleotide
ccggatggtcactctttaggaag

SEQ ID NO: 35 - DNA, 20 bp, Artificial Sequence
  synthetically generated oligonucleotide
ttgctccaaactggcgtcta

SEQ ID NO: 36 - DNA, 21 bp, Artificial Sequence
  synthetically generated oligonucleotide
acgtgatctccgtgtccttgt

SEQ ID NO: 37 - DNA, 21 bp, Artificial Sequence
  synthetically generated oligonucleotide
ctgccagtccgaaaatggaac

SEQ ID NO: 38 - DNA, 20 bp, Artificial Sequence
  synthetically generated oligonucleotide
cttcatccactggggctatc

SEQ ID NO: 39 - DNA, 23 bp, Artificial Sequence
  synthetically generated oligonucleotide
gacagagttagtgaatggagacc

SEQ ID NO: 40 - DNA, 21 bp, Artificial Sequence
  synthetically generated oligonucleotide
aaaagttcggagagtgtaggc

SEQ ID NO: 41 - DNA, 18 bp, Artificial Sequence
  synthetically generated oligonucleotide
gagaagcccagccagtcg

SEQ ID NO: 42 - DNA, 18 bp, Artificial Sequence
  synthetically generated oligonucleotide
ctcttgctctgggcttca

SEQ ID NO: 43 - DNA, 17 bp, Artificial Sequence
  synthetically generated oligonucleotide
cctgcgacccacacaag

SEQ ID NO: 44 - DNA, 18 bp, Artificial Sequence
  synthetically generated oligonucleotide
gacccaccgaagacacag

SEQ ID NO: 45 - DNA, 21 bp, Artificial Sequence
  synthetically generated oligonucleotide
ccagcagcatgatcaaaacac

SEQ ID NO: 46 - DNA, 22 bp, Artificial Sequence
  synthetically generated oligonucleotide
ggtggctacatgttagagtgtc

SEQ ID NO: 47 - DNA, 22 bp, Artificial Sequence
  synthetically generated oligonucleotide
atcatagccataggacatctgg

SEQ ID NO: 48 - DNA, 18 bp, Artificial Sequence
  synthetically generated oligonucleotide
ctggacagcctggacttc

SEQ ID NO: 49 - DNA, 21 bp, Artificial Sequence
  synthetically generated oligonucleotide
ctctgagtgatcctctggttc

SEQ ID NO: 50 - DNA, 23 bp, Artificial Sequence
  synthetically generated oligonucleotide
ccataagaacaagaccacatcct

SEQ ID NO: 51 - DNA, 20 bp, Artificial Sequence
  synthetically generated oligonucleotide
cttgctggtgttggtgattc

SEQ ID NO: 52 - DNA, 22 bp, Artificial Sequence
  synthetically generated oligonucleotide
atcagcctctgaatcatgtgaa

SEQ ID NO: 53 - DNA, 21 bp, Artificial Sequence
  synthetically generated oligonucleotide
tgctttttccaggggtgtgtt

SEQ ID NO: 54 - DNA, 23 bp, Artificial Sequence
  synthetically generated oligonucleotide
ttacttcctgcactaatttggca